European Patent Specification EP 4 225 347 B1, published December 25, 2024. Title: CONNEXIN 43 FOR USE IN THE TREATMENT OF A CANCER TYPE CHARACTERIZED BY THE ACTIVATION OF A MITOGEN-ACTIVATED PROTEIN KINASE. Applicant: Fundación Profesor Novoa Santos SERVIZO GALEGO DE SAÚDE. The sequence listing filed with the application follows.

SEQUENCE LISTING (4 sequences)

SEQ ID NO: 1 - DNA, 20 bp, Artificial sequence
  Artificial sequence
acatgggtgactggagcgcc

SEQ ID NO: 2 - DNA, 20 bp, Artificial sequence
  Artificial sequence
atgatctgcaggacccagaa

SEQ ID NO: 3 - DNA, 22 bp, Artificial sequence
  Artificial sequence
ttgagtttggaaacatctggag

SEQ ID NO: 4 - DNA, 21 bp, Artificial sequence
  Artificial sequence
gcccaaagggaactgatagtc